European Patent Application EP 4 299 764 A1, published January 3, 2024. Title: METHODS FOR DETECTING PANCREATIC CANCER USING DNA METHYLATION MARKERS. Applicant: Universal Diagnostics, S.A. Application EP. The sequence listing filed with the application follows.

SEQUENCE LISTING (25 sequences)

SEQ ID NO: 1 - DNA, 302 bp, Homo sapiens
  source 1..302: mol_type = other DNA
gcatctttccgagctccgggcgctcgctcccgggccggagccgcagcgacgctggcgggagcctgccagaggggctgaggcggggcttgccgctccccacctccctacgaggcggggtctacatgcccctctcgctgcaacgcggccaaccgcaggcgggtgctgacgacacctccacccccggctcgtaagctaatttgcgtcacatatggcgtaagagccctgtcggagcgggggacctacctagcccatccctcctccatcaaatagtaggcgcctcgctagaattcccacttggcccc

SEQ ID NO: 2 - DNA, 302 bp, Homo sapiens
  source 1..302: mol_type = other DNA
gagatccagttcctgcgaactgtaagcgccgtgcgtcgcgtgtgctgtcaggggaagggggcgtcagggcatccactagcggggtccgggcagagtgacagcgggcagcggggactcgcgggcggggcgagggggtgccccctgaggatgcgggaggagcgggcatcaccaagtgtgtgcaggtgtgcgtgttggggcgagggaaggcaagggcgcgtgtctgtgcgcgcgtgtggaaagctagaggatggagcgcggctagccggcggcaggcgcccgggctcggacccggggcaccgggg

SEQ ID NO: 3 - DNA, 302 bp, Homo sapiens
  source 1..302: mol_type = other DNA
tcaaatttgtcaatgttcatgtcatttttgctttaggtcacagagcaaggtgcaaattcctggcatctttactagttgcagccaatttcggcgatttcggcggtgacggggattctcagaggagccgcgtgcccgtgcgctcccgcctgtcggccccagagagcgcagccctgacacctcctcccggaagcccgccggcccgaccctggtttggaaggagaggctcagggagtgggacagagggtatctctctttccccagcgtccacccccagacgcctcctacccccaaccagggaggtt

SEQ ID NO: 4 - DNA, 302 bp, Homo sapiens
  source 1..302: mol_type = other DNA
ggaagagagaaagcaagagagcgggagggtgcgcggagcggagcggagacagagctcgcgggcatggggtgagagcgggaggaagcagaggcagaggcggagcaggggcgcaggtgcctgcaacccaggatcccggggcgctaaaggcttcgggttctaccgcacgctcagtcgctggctccagaggtgctgctgggggccagggttcactgccgcgcgccaggtgcctgcccgtgaggcggcgcggggctcccgggtggctgcgcgcccagacgcctgcccgggaggccgcctgaggctcc

SEQ ID NO: 5 - DNA, 302 bp, Homo sapiens
  source 1..302: mol_type = other DNA
gctggcggcaggagccctgggtcctccccaggagagggacccagagcccagaccaagtccaacccgccaacctgcgccacccatgcgcgcactgggggctgcagagccccgccaggctgcccgcggccgggagcgtaaggccggggtccacgcctcgattttcagtgtccgcagcccctaccccgcctatctgcgacgcaaggcgaaaccttgtttttgcggaaaatgcctggctttgtctagggctggggtgggggcgtctgggcagccaccctcggccacattaaaattcctggcgcccc

SEQ ID NO: 6 - DNA, 302 bp, Homo sapiens
  source 1..302: mol_type = genomic DNA
cttcaaaccgcgccatcctcctgggtcttccctctcggagcgcaagggctgggtcccccaaggagaccccgggtgcgaagtcgcagaggagagggcgtctcggggaggccagggacaggtctgcgacgaagtccagcaccgtagtgtccacgcagctctccggataggccgccatcgcttcggcttggccctgcctctcatcggttttccgcagggaggggcgaggttgctggtggggattcttaacagccttgaatctgatggggcaccatcaccgaaaggccagggaacattaaatattt

SEQ ID NO: 7 - DNA, 302 bp, Homo sapiens
  source 1..302: mol_type = genomic DNA
acaggggaagggtgttctttctctctgccctccctttccatctccagctccccatttcctttctcacctcctcctccactccctgcctcttctccccacccatcctggcgggcgggctgcgcggaggctcgggagctggccggggaggggcggatggaggggcctgggttgccagctcccttggtcggggtcctgctcgctggggcttgtgtgttctctgcggcgggccgcgtccccgctgagcctcgcggtgacagccgcctttggcagcgagcgctcggggcacttctatccccgcctct

SEQ ID NO: 8 - DNA, 302 bp, Homo sapiens
  source 1..302: mol_type = genomic DNA
tgagaaacgcgtccgcggcagctactgagggtctgccccacctttagcttcaggttgacaactgccttcagcgcgttctcagctcagctggccctatgggtcccctaaaatcgcccgagcgtccgccctgtctgacctgcccccctgccgcggcgcacatttcagcttttcagcttcacggtggagctcgcagtaattgagtcgcgagggttatttttcctggcctcacctcgcggtcctgagcctgcagggagctttcggaaagacatcgccccctccccctgagtccccggcagcttctg

SEQ ID NO: 9 - DNA, 302 bp, Homo sapiens
  source 1..302: mol_type = genomic DNA
cccggcgaggaggcgcggaaccatggccgatgggggcgagggcgaagacgagatccagttcctgcgaactgtaagcgccgtgcgtcgcgtgtgctgtcaggggaagggggcgtcagggcatccactagcggggtccgggcagagtgacagcgggcagcggggactcgcgggcggggcgagggggtgccccctgaggatgcgggaggagcgggcatcaccaagtgtgtgcaggtgtgcgtgttggggcgagggaaggcaagggcgcgtgtctgtgcgcgcgtgtggaaagctagaggatggag

SEQ ID NO: 10 - DNA, 302 bp, Homo sapiens
  source 1..302: mol_type = genomic DNA
ggctgagtttagccggcgggagcctggagtccgctcggcacgagcgcggggacgcgggagccgcgcgggacccaagcagtttttccgagcagccgccaggctcagccccgctcccagcctcgctgcgcagccagagacctgctatggccacgtctatactcggggtaagtcgcaagcgcggcaacgcatttgcttgttttaaccggagtaatttttcgttatggcttctggggtctgcggctccggagaaactgttgctgctagactgcagcttcagcttctattagcactttccacatttc

SEQ ID NO: 11 - DNA, 302 bp, Homo sapiens
  source 1..302: mol_type = genomic DNA
aaggagcgcaaggagtaggggactgaaggtgcccaaagctagtgggtcagtgtcactttcttcctccctttcgcccctttcctcccgctcctttctcccctgtggtctctgctcagcacccctttctctccagccccgactgcccatcttcgcccctaccctcgcgcgtcggggccgtgtctacacccaccccaggacctggtccgtccaggctccttcccatcctcacacccgcgcctttctccctgcggccccggctcgctgctccagctgcccagctcttcccaggacaggggatcccg

SEQ ID NO: 12 - DNA, 302 bp, Homo sapiens
  source 1..302: mol_type = genomic DNA
caccggcactgcgcgcgtcctcttcgcttccgcgccgcccccgccaggtggagggggtggggacggtcgggacaggcgggagtttagaggagggagccgcagaaggggttccccgcttgagctaacgtagtggtggcatccagaggtgaacgcgggagcggccgcctgcggagggcacccggctgcgtggcgtccgctcgggccgctgctgcggcagaggtgccctggttgggcggctgggcgcctggggttcgacgccggccgggatccctgggtgtgcgcggagatgcgcgccgcggagg

SEQ ID NO: 13 - DNA, 302 bp, Homo sapiens
  source 1..302: mol_type = genomic DNA
accccacctcttcgatttcaaagcacttaaaaatagtactctggcgtgcgagcggcttctaggacacggtgatttcctcctgttcctcgccctcctcttcctcctcggaatctgagaagtccgaaggtttcccgggactgctcgagtgcgcgggcgaggggggcagcggccctggcagccgcgggtcccgcaggtgctgggggtcggaggacgcgtggtaggccaggcggtggctggggctgcccgggccctcctcctcctcttcgttcccagggcccttctggcccacgtcgctgaggtcc

SEQ ID NO: 14 - DNA, 302 bp, Homo sapiens
  source 1..302: mol_type = genomic DNA
aagactggaagatgtctccttatatacaccactctttcaaattctcatttgtagctcccggaactcagaagacagtcgacccccaaaactgtccaggaagtaatcggtttccggcttttggacaatggtccctcgcttaacgaatgctaacgaatgctcccttagctgggagctgcagggaccggtcccggcaggtctaaccaaccgtccgcaggcgccgtggtcgagagcagagccgagacggcggggcagggtgccaagcggagggcacagcctggcagccaccgttggcggcaggagag

SEQ ID NO: 15 - DNA, 302 bp, Homo sapiens
  source 1..302: mol_type = genomic DNA
agttgctctccggagtccaacacgcgcgcaggcaaaccccacctccctccttcgaccccaacagaattttttttaaattttaatccacagggggtatttcctttcctgtttacccgagcgaagagtggcccccggtggcccaaggaggggcgcctccaggcgcagggctccggcggctccagctgctcccgggctggctagcgggcgctggcgcaggcggcgccggggtggcggggctgcggagcccgggacgcgggcagaggcggctcggagccccccgggcgggtggccgggctcgctgg

SEQ ID NO: 16 - DNA, 302 bp, Homo sapiens
  source 1..302: mol_type = genomic DNA
agagggtaccagggatttcccagacccccaccagccctcaggaatagcgtagagagaggaacgtcgcctggctgagaaaggtggatgggcatacccatgtacctttgtgtattaagtacccacaacctccgaacttagccgtccctgtcccggcccgcccaactgctgccgccgcatctgcagaaaccactcgtgttgaggcctcggagcagccgggagcaccacgctggagcaaaaaagccggagggcgcagggctccagcccggctgaccatcccacccagcgcagggaccaacggaaaa

SEQ ID NO: 17 - DNA, 302 bp, Homo sapiens
  source 1..302: mol_type = genomic DNA
gaggcggggagggaggcgggagggggaggggacggtgtggatggccccgaggtccaaaaagaaagcgcccaacggctggacgcacaccccgccaggcctcctggaaacggtgccggtgctgcagagcccgcgaggtgtctgggagttgggcgagagctgcagacttggaggctcttatacctccgtgcaggcggaaagtttgggggcagcagtgtcattggcctgacgtgaggaggagggacttttcgaagttttataggaaagtttccgctttccagtccccctcccccgtcccacctccc

SEQ ID NO: 18 - DNA, 302 bp, Homo sapiens
  source 1..302: mol_type = genomic DNA
tctcctgacagctccaggaaaggcagaccccttccccagccagccaggtaaggtaaagactgctgttgagcttgctgttactgagggcgcacagaccctggggagaccgaagcttgccactgcgggattctgtggggtaacctgggtctacggaagtttcctgaaagaggggagaagggtttgcatttttcctatggaggattcttctctctctagcatttcgtttgatgtattcaactggtagaagtgagatttcaacaggtagcagagagcgctcacgtggaggaggtttggggcgccgc

SEQ ID NO: 19 - DNA, 302 bp, Homo sapiens
  source 1..302: mol_type = genomic DNA
ccggccgcgccgagaactaaatccgcgggctgaaattacgttttaaaaattaacatgttgaagcgtgtgccatttagtgagaggtgttttgggcaaagaatcaatttaactgtgactgaccgacgggcttgactgtattaattctgctaccgaaaaaaaaaaaaaaaaaaaagcaatgagccgcaagccttggactcgcagagctgccggtgcccgtccgagagccccaccagcgcggctcacgcctcagtctcgccgccccaaggtgggatccgacgcccaaaggagggcgccccaaggtg

SEQ ID NO: 20 - DNA, 302 bp, Homo sapiens
  source 1..302: mol_type = genomic DNA
ttccccgcttgagctaacgtagtggtggcatccagaggtgaacgcgggagcggccgcctgcggagggcacccggctgcgtggcgtccgctcgggccgctgctgcggcagaggtgccctggttgggcggctgggcgcctggggttcgacgccggccgggatccctgggtgtgcgcggagatgcgcgccgcggaggcgaatggagggaggaggagaaggagaaagaggagaaagaggagaaggaggaggaggaggaggagggcgaagcggcaagcgcggggcgcaggcggaccggcggccgggc

SEQ ID NO: 21 - DNA, 302 bp, Homo sapiens
  source 1..302: mol_type = genomic DNA
tttcttattacctttgattactcctttttaccaaatttctggaggagctcagtggggaggattggggggaatctgattttaagaaagaaagcaccgaaggggcaattattaattttcctcgggtttggaatcaccctctggacaagagaacgggcgagcgggagctaggagggaagagtggagaggaccggcgaggcgcgccagccggagccacctccttcccggccgccccctccccactccccctacacacacacgctcgctcgctcgccggcgcgcgcacaccccccgcgccggacccg

SEQ ID NO: 22 - DNA, 302 bp, Homo sapiens
  source 1..302: mol_type = genomic DNA
tacattctgcttcggtttcttcagggctccctgaggccaccggatgcttttcccccgtgcttacttgcccaccaaaagaggggaaaaggtgggtgcacagcgggttctcagagggtgctcctgagccccctggagctccgggtactcggccggccggcggccactcggcagcgctgcgggctgccgggaactgttctccgctcggggtgctgaaagcggacgcgggagagcgcgcagagaaggcgaggagccgggtcggccaggctctcctgcaggcgcgggtcctgctcgcggggcgtctc

SEQ ID NO: 23 - DNA, 302 bp, Homo sapiens
  source 1..302: mol_type = genomic DNA
gtggcgagtgaagtggagcagtgcattcgtgtcatcacccacccgaccccggctgcgctcctccgaccccgccgcctactcccgccgaggaggaggagcacgtgcggtcggtggggcgcagggccggggagccaggggggtgccggggctcgaggccgcggggccgcgggggccgcgctctgctctccgcccaggctgggccactggagcgcgggagccctggagcccggcgctgcccggcgctacccgccgccctcgggacagtcaccgtgagcaaaagagtcggtgtcatgtgcgtaaac

SEQ ID NO: 24 - DNA, 302 bp, Homo sapiens
  source 1..302: mol_type = genomic DNA
cagagcagcccctaccctccaatattttgcaggaggggagaagaggaaaaagagaactggatatttgatatgtcgaaagaatgatcgatgatgaggctgcaccgtaggagcttgccggtctccgaccgctgctggcctgcgaagccggcacgtttacaaggctcagccctgggctgtcatacttccaccagaacagcagcaaatgcgttcatggcgaattattttgcagacgtgagaactctgatttttttttcagcttctaggacttacacacagttagcctgggtcttttttagcacatt

SEQ ID NO: 25 - DNA, 302 bp, Homo sapiens
  source 1..302: mol_type = genomic DNA
ccgtgttacggccgcctaccggctgcagaggagaagggtaggctgtgggcggcggcggggcgcggaggggtagccaggagcgcaggctgggctccgcacctccctgccccaaaacccattgatgcagcggccactgcggctgccgagcggcgtcttcccagagcccggggctgtgcccgcccgatgcaggatgcaactgaggaagcccgctccaaagcaaaacaaaacaaattcctccagccatgccgtctttctccaacccactcaagcgaaagaatggacaccagttaccagccgctgac